European Patent Application EP 4 163 394 A1, published April 12, 2023. Title: METHOD FOR DETERMINING TOUGH AND DRY MEAT SYNDROME (TDMS). Applicant: Université de Liège. Application EP. The sequence listing filed with the application follows.

SEQUENCE LISTING (7 sequences)

SEQ ID NO: 1 - RNA, 3516 nt, Bos taurus
  source 1..3516: mol_type = mRNA; note = bovine ATPase sarcoplasmic/endoplasmic reticulum Ca2+ transporting 1 (ATP2A1)
gaacgggggtcagagcttcgtggagggaagaataacctgggggggggaaggaaagaaaaaggaagaaacccagacaaacaggcaggtggacacactgaggaaggcccccgacgtgtgagaacccccccagaaggaacacaccgccccctggcccccaggaagggagcaccatggaggctgcgcactccaagaccacagaagaatgtttggcctattttggggtgagcgaaactacaggcctcaccccggaccaagttaagcggcatctggagaaatatggccataatgagctccctgctgaggaggggaagtccctgtgggagctggtgttagagcagtttgaagacctcctggtgcggatccttctcctggccgcctgcatttcctttgtgctggcctggtttgaggaaggcgaagagactgtcaccgcctttgttgaaccctttgtcatcctcttgatcctcattgccaatgccatcgtgggggtttggcaggagcggaatgcagagaatgccatcgaggctctgaaggaatatgaacccgagatggggaaggtctaccgggctgaccgcaagtcagtacaaaggatcaaagctcgggatattgttcctggagacatcgtggaggtggctgtgggggacaaggtcccggcagatatccgcatcctcaccatcaagtctaccaccctccgggtcgaccagtccatcctgacaggcgagtctgtctctgtcatcaagcacacagaacctgttcccgacccccgagctgtcaaccaggataagaagaacatgcttttctcgggcaccaacatcgcagccggcaaggccatcggcattgtggccaccaccggtgtgggcaccgagattgggaagatccgtgaccaaatggccgccacagagcaggacaagacccctctgcagcaaaagctggatgagtttggggagcagctctccaaggtcatctccctcatctgcgtggccgtctggctcatcaacattggccacttcaacgaccccgtgcatgggggctcctggatccgtggtgccatctactactttaagatcgccgtggccctggctgtggctgccatccccgagggccttcctgcagtcatcaccacctgcctggccttgggcacccgccggatggcaaagaagaacgcgatcgtgaggagcctgccctccgtggagactctgggctgcacctctgtcatctgttccgacaagacgggcaccctcaccaccaaccagatgtctgtctgcaagatgttcatcatcgacaggatagatggggacctctgcctgctgaacgagttctctgtcactggctccacttacgctcctgaaggagaggtcttgaagaatgataagccagtccgctcagggcagtatgacgggctggtggagctggccaccatttgtgccctctgcaatgactcctccttggacttcaatgagaccaaaggtatttatgagaaggtgggagaggccaccgagacagccctcaccaccctggtggagaagatgaatgtattcaacactgaagtgagaaacctctcgaaggtagagagggccaacgcctgcaactcggtgatccgccagctaatgaagaaggaattcaccctggagttctcccgggaccgaaagtccatgtctgtctattgctctccagcaaaatcccgggctgctgtgggcaataagatgtttgtcaagggtgcccctgagggggtcatcgatcgctgtaactacgtgcgagtgggcaccacccgggtgcccatgacagggccggtgaaggagaagattctgtcggtgatcaaagagtggggtactggccgggacaccctgcgctgcctggcgctggccactcgggacaccccccccaagcgagaggagatggtcctggatgactctaccaagttcatggagtacgagacggacttgacattcgttggcgtcgtgggcatgctggacccgccccgcaaggaggtcatgggctccatccaactatgccgagacgctggaatccgagtaatcatgatcaccggagacaacaagggcacggccattgccatctgccgacggattggcatcttcggggagaacgaggatgtggctgaccgggcctacactggccgggagttcgatgacctgcccctggccgagcagcgggaggcctgccgacgcgcctgctgcttcgcccgcgtggagcccacccacaagtcgaagatcgtggagtatctgcagtccttcgatgagatcacggcgatgacaggtgatggcgtcaatgacgcccctgcgctgaagaaggcggaaatcggcattgccatgggatccggcactgccgtggccaagacagcctctgagatggtgctggccgacgacaacttctccaccattgtggctgccgtggaggagggccgggccatctacaacaacatgaagcagtttatccgctacctcatctcctccaacgtgggcgaggtggtctgcatcttcctgacagctgccctggggctgcccgaggccctgatccctgtgcagctgctgtgggtgaacctggtgaccgatgggctcccagccacagccctgggcttcaaccccccagacctggacatcatggaccggcccccccggacccccaaggagcccctcatcagtggctggctcttcttccgctacatggcaattgggggctatgtgggtgcagccaccgtgggagcagcggcctggtggttcctgtatgctgaggacgggcctcacgtcacctacagccagctgactcacttcatgaagtgctcggagcacagcccagacttcgagggtgtggactgtgaggtcttcgaggccccgcagcccatgaccatggccttgtctgtgctggtcaccatcgagatgtgcaatgctctcaacagcctgtctgagaatcagtccctcgtgcggatgccaccctgggtgaacatctggctggtgggctccatcggcctctccatgtccctccacttcctcatcctctacgtggaccctctgccgatgatcttcaagctccaagccctggacctgtaccattggctcatggtcctcaagatctcattaccagtcattgggctcgacgaaatcctcaagttcgttgctcgaaactacctggagggataacccgtttccccctcctccatctctttgaaccgtgtcacagatccagaagatgaaagaaggaagcaaccaggccttttgccctccctccccaccccatagtgacgcatcttcggccagagctgtggcacaggccccaccctccacaacgttccctattcctcccgcccgacattcttgtttataaacactatgtccccttcacttctcctcccccctcagcaacctgtcccccttttgcccttgtgaaacctcccctccccgaccccgtggggctcgcagggacaaggcgactgattgagctgagctgcttatttattgaaaataaatgacagaaaaatcaaaaaaaaaaaaaaaaaaaaaaaaa

SEQ ID NO: 2 - protein, 993 aa, Bos taurus
  source 1..993: note = ATP2A1 protein
MEAAHSKTTEECLAYFGVSETTGLTPDQVKRHLEKYGHNELPAEEGKSLWELVLEQFEDLLVRILLLAACISFVLAWFEEGEETVTAFVEPFVILLILIANAIVGVWQERNAENAIEALKEYEPEMGKVYRADRKSVQRIKARDIVPGDIVEVAVGDKVPADIRILTIKSTTLRVDQSILTGESVSVIKHTEPVPDPRAVNQDKKNMLFSGTNIAAGKAIGIVATTGVGTEIGKIRDQMAATEQDKTPLQQKLDEFGEQLSKVISLICVAVWLINIGHFNDPVHGGSWIRGAIYYFKIAVALAVAAIPEGLPAVITTCLALGTRRMAKKNAIVRSLPSVETLGCTSVICSDKTGTLTTNQMSVCKMFIIDRIDGDLCLLNEFSVTGSTYAPEGEVLKNDKPVRSGQYDGLVELATICALCNDSSLDFNETKGIYEKVGEATETALTTLVEKMNVFNTEVRNLSKVERANACNSVIRQLMKKEFTLEFSRDRKSMSVYCSPAKSRAAVGNKMFVKGAPEGVIDRCNYVRVGTTRVPMTGPVKEKILSVIKEWGTGRDTLRCLALATRDTPPKREEMVLDDSTKFMEYETDLTFVGVVGMLDPPRKEVMGSIQLCRDAGIRVIMITGDNKGTAIAICRRIGIFGENEDVADRAYTGREFDDLPLAEQREACRRACCFARVEPTHKSKIVEYLQSFDEITAMTGDGVNDAPALKKAEIGIAMGSGTAVAKTASEMVLADDNFSTIVAAVEEGRAIYNNMKQFIRYLISSNVGEVVCIFLTAALGLPEALIPVQLLWVNLVTDGLPATALGFNPPDLDIMDRPPRTPKEPLISGWLFFRYMAIGGYVGAATVGAAAWWFLYAEDGPHVTYSQLTHFMKCSEHSPDFEGVDCEVFEAPQPMTMALSVLVTIEMCNALNSLSENQSLVRMPPWVNIWLVGSIGLSMSLHFLILYVDPLPMIFKLQALDLYHWLMVLKISLPVIGLDEILKFVARNYLEG

SEQ ID NO: 3 - protein, 46 aa, Bos taurus
  source 1..46: note = ATP2A1 exon 5 protein
ERNAENAIEALKEYEPEMGKVYRADRKSVQRIKARDIVPGDIVEVA

SEQ ID NO: 4 - protein, 46 aa, Bos taurus
  source 1..46: note = ATP2A1 exon 5 protein R143W variant
ERNAENAIEALKEYEPEMGKVYRADRKSVQRIKAWDIVPGDIVEVA

SEQ ID NO: 5 - protein, 46 aa, Felis catus
  source 1..46: note = ATP2A1 exon 5 protein
ERNAENAIEALKEYEPEMGKVYRADRKTVQRIKARDIVPGDIVEVA

SEQ ID NO: 6 - protein, 46 aa, Gallus gallus
  source 1..46: note = ATP2A1 exon 5 protein
ERNAESAIEALKEYEPEMGKVIRADRSGVQRIRARDIVPGDIVEVA

SEQ ID NO: 7 - protein, 46 aa, Danio rerio
  source 1..46: note = ATP2A1 exon 5 protein
ERNAESAIEALKEYEPEMGKVYRSDRKSVQRIKAREIVPGDIVEVS